European Patent Application EP 4 365 202 A1, published May 8, 2024. Title: ANTI-TROP2 SINGLE-DOMAIN ANTIBODY AND USE THEREOF. Applicant: NANOMAB TECHNOLOGY LIMITED. The sequence listing filed with the application follows.

SEQUENCE LISTING (55 sequences)

SEQ ID NO: 1 - protein, 124 aa, Camelus bactrianus
QVQLQESGGGSVLAGGSLRLSCTVSGSFVSSRSMAWFRQTPGKEREGVAAISQYGDPKYAGSVKGRFTMSRDNAKNTLLLQMNSLKPEDTAIYYCAAGEAWELATLSRSDYIYWGQGTQVTVSS

SEQ ID NO: 2 - protein, 123 aa, Camelus bactrianus
QVQLQESGGGSVQAGGSLRLSCVVSGYTTTRYSMAWFRQAPGKEREGVAGIDTDVLTTYKPSVEGRFTISRDSAKRTLYLQMNSLKPEDTAMYYCATGTGNFLALDPVWYNTWGQGTQVTVSS

SEQ ID NO: 3 - protein, 126 aa, Camelus bactrianus
QVQLQESGGGSVQAGGSLRLSCAVSGLTSSTTCMGWFRQAPGKEREGVAVIRSSGETTAADSVKGRFTISRDNAKNTLSLQMTSLKPEDTAMYYCAAAWPYSGCLLPLSSGDFTYWGQGTQVTVSS

SEQ ID NO: 4 - protein, 125 aa, Camelus bactrianus
QVQLQESGGGSVQAGGSLKLSCVVSGYTVSSVCMAWFRQAPGMERELVAGFYHSGGTYYGDSVKGRFTASQDNAKNTLYLQMNSLKPEDTATYYCARARYPSSACGTSPSNYNIWGQGTQVTVSS

SEQ ID NO: 5 - protein, 114 aa, Camelus bactrianus
QVQLQESGGGSVQAGGSLRLSCAASGFSVSTTWMHWVRQAPGKGLEWVSRIAINDHTFYAESVKGRFTMSTDNAKNTVYLQMTSLKPEDTAVYYCSPYSDYRIRGQGTQVTVSS

SEQ ID NO: 6 - protein, 125 aa, Camelus bactrianus
QVQLQESGGGSVQPGGSLRLSCVVSGYTVSSVCMAWFRQAPGMERELVAGFYHSGGTYYGDSVKGRFTASQDNAKNTLYLQMNSLKPEDTATYYCARARYPSSACGTSPSNYNIWGQGTQVTVSS

SEQ ID NO: 7 - protein, 125 aa, Camelus bactrianus
QVQLQESGGGSVQPGGSLRLSCVASGYTASSVCMAWFRQAPGKERELVAGYYHSGGTYYGDSVKGRFTASQDNAKNTLYLQMNSLKPEDTATYYCARARYPSSACGTSPSNYNIWGQGTQVTVSS

SEQ ID NO: 8 - protein, 130 aa, Camelus bactrianus
QVQLQESGGGSVQAGGSLRLSCAASGFPYSSYSMGWFRQAPGKEREGVAAIYTGGGSTYYAGSVKGRFTISQEHATNTLYLQMNSLKPEDTAMYYCAANMVDNGVISGIQALGVRYYNYWGQGTQVTVSS

SEQ ID NO: 9 - DNA, 372 bp, Camelus bactrianus
caggtgcagctgcaggagtctggaggaggctcggtgctggctggagggtctctgagactctcctgtacagtctctggatcgttcgtcagcagccgctccatggcctggttccgccagactccagggaaggagcgcgagggggtcgcagctatttctcagtatggggacccaaagtacgcaggctccgtgaagggccgattcaccatgtctcgagacaacgccaagaacactctcttgctacaaatgaacagcctgaaacctgaggacactgccatctactactgtgcggcaggcgaggcttgggagttggctacgttgtccaggagcgactatatctactggggccaggggacccaggtcaccgtctcctca

SEQ ID NO: 10 - DNA, 369 bp, Camelus bactrianus
caggtgcagctgcaggagtctgggggaggctcggtgcaggctggagggtccctgagactctcctgtgtagtctctggatacaccaccacccggtactccatggcttggttccgccaggctcctgggaaggagcgcgagggggtcgcaggtattgatactgatgttcttacaacctacaaaccgtctgttgagggccgattcaccatctcccgagacagcgccaagagaactctgtatctgcaaatgaacagcctgaaacctgaggacactgccatgtactactgtgcgacagggactggaaatttcttggcactggatccggtctggtataatacctggggccaggggacccaggtcaccgtctcctca

SEQ ID NO: 11 - DNA, 378 bp, Camelus bactrianus
caggtgcagctgcaggagtctgggggaggctcggtgcaggctggagggtctctgagactctcctgtgcagtctctggactcaccagcagtaccacctgcatgggctggttccgacaggctccagggaaggagcgcgagggggtcgcagttattagaagttctggtgagacaaccgccgcagactccgtgaagggccgattcaccatctcccgagacaacgccaagaacactctgtctttgcaaatgaccagcctgaaacctgaggacactgccatgtactactgtgcggcagcgtggccgtatagtggttgcctactccccctgtcgtcgggggactttacttactggggccaggggacccaggtcaccgtctcctca

SEQ ID NO: 12 - DNA, 375 bp, Camelus bactrianus
caggtgcagctgcaggagtctgggggaggctcggtgcaggctggagggtctctgaaactctcctgtgtagtctctggatacaccgttagtagcgtctgcatggcctggttccgccaggcgccagggatggagcgcgaactggtcgcaggtttttatcatagtgggggcacttactatggcgactccgtgaagggccgattcaccgcctcccaagacaacgccaagaacacgctgtatctgcaaatgaacagcctgaaacctgaggacactgccacatactactgtgcgcgcgcacgttacccgtcatctgcctgcggcacttcaccatcaaattataacatctggggccaggggacccaggtcaccgtctcctca

SEQ ID NO: 13 - DNA, 342 bp, Camelus bactrianus
caggtgcagctgcaggagtctgggggaggctcggtgcaggctggagggtctctgagactctcctgtgcagcctctggattcagcgtcagtaccacctggatgcactgggtccgccaggctccagggaaggggcttgagtgggtctcgcgtattgctattaatgatcacacattctatgcagagtcagtgaagggccgattcaccatgtccacagacaacgccaagaatacggtgtatctgcaaatgaccagcctgaaacctgaggacacggccgtgtattactgtagtccatatagtgactatcgaattcgtggccaggggacccaggtcaccgtctcctca

SEQ ID NO: 14 - DNA, 375 bp, Camelus bactrianus
caggtgcagctgcaggagtctgggggaggctcggtgcagcctggagggtctctgagactctcctgtgtagtctctggatacaccgttagtagcgtctgcatggcctggttccgccaggcgccagggatggagcgcgaactggtcgcaggtttttatcatagtgggggcacttactatggcgactccgtgaagggccgattcaccgcctcccaagacaacgccaagaacacgctgtatctgcaaatgaacagcctgaaacctgaggacactgccacatactactgtgcgcgcgcacgttacccgtcatctgcctgcggcacttcaccatcaaattataacatctggggccaggggacccaggtcaccgtctcctca

SEQ ID NO: 15 - DNA, 375 bp, Camelus bactrianus
caggtgcagctgcaggagtctgggggaggctcggtgcagcctggagggtctctgagactctcctgtgtagcctctggatacaccgcgagtagtgtctgcatggcctggttccgccaggcgccagggaaggagcgcgaactggtcgcagggtattatcatagtgggggcacttactatggcgactccgtgaagggccgattcaccgcctcccaagacaacgccaagaacacgctgtatctgcaaatgaacagcctgaaacctgaggacactgccacatactactgtgcgcgcgcacgttatccgtcatctgcctgcggcacttcaccatcaaattataacatctggggccaggggacccaggtcaccgtctcctca

SEQ ID NO: 16 - DNA, 390 bp, Camelus bactrianus
caggtgcagctgcaggagtctggaggaggctcggtgcaggctggagggtctctgagactctcctgtgcagcctctggatttccctacagtagctactcgatgggctggttccgccaggctccagggaaggagcgcgagggggtcgcagctatttatactggtggtggtagcacatactatgccggctccgtgaagggccgattcaccatctcccaagagcacgccacgaacacactgtatctgcagatgaacagcctgaaacctgaggacactgccatgtactactgtgcggcaaatatggtagataacggcgttatctctggtattcaggctcttggtgttaggtactataactactggggccaggggacccaggtcaccgtctcctca

SEQ ID NO: 17 - protein, 10 aa, Camelus bactrianus
GSFVSSRSMA

SEQ ID NO: 18 - protein, 10 aa, Camelus bactrianus
GYTTTRYSMA

SEQ ID NO: 19 - protein, 10 aa, Camelus bactrianus
GLTSSTTCMG

SEQ ID NO: 20 - protein, 10 aa, Camelus bactrianus
GYTVSSVCMA

SEQ ID NO: 21 - protein, 10 aa, Camelus bactrianus
GFSVSTTWMH

SEQ ID NO: 22 - protein, 10 aa, Camelus bactrianus
GYTASSVCMA

SEQ ID NO: 23 - protein, 10 aa, Camelus bactrianus
GFPYSSYSMG

SEQ ID NO: 24 - protein, 8 aa, Camelus bactrianus
AISQYGDP

SEQ ID NO: 25 - protein, 8 aa, Camelus bactrianus
GIDTDVLT

SEQ ID NO: 26 - protein, 8 aa, Camelus bactrianus
VIRSSGET

SEQ ID NO: 27 - protein, 8 aa, Camelus bactrianus
GFYHSGGT

SEQ ID NO: 28 - protein, 8 aa, Camelus bactrianus
RIAINDHT

SEQ ID NO: 29 - protein, 9 aa, Camelus bactrianus
AIYTGGGST

SEQ ID NO: 30 - protein, 16 aa, Camelus bactrianus
GEAWELATLSRSDYIY

SEQ ID NO: 31 - protein, 15 aa, Camelus bactrianus
GTGNFLALDPVWYNT

SEQ ID NO: 32 - protein, 18 aa, Camelus bactrianus
AWPYSGCLLPLSSGDFTY

SEQ ID NO: 33 - protein, 17 aa, Camelus bactrianus
ARYPSSACGTSPSNYNI

SEQ ID NO: 34 - protein, 6 aa, Camelus bactrianus
YSDYRI

SEQ ID NO: 35 - protein, 21 aa, Camelus bactrianus
NMVDNGVISGIQALGVRYYNY

SEQ ID NO: 36 - protein, 25 aa, Camelus bactrianus
QVQLQESGGGSVLAGGSLRLSCTVS

SEQ ID NO: 37 - protein, 25 aa, Camelus bactrianus
QVQLQESGGGSVQAGGSLRLSCVVS

SEQ ID NO: 38 - protein, 25 aa, Camelus bactrianus
QVQLQESGGGSVQAGGSLRLSCAVS

SEQ ID NO: 39 - protein, 25 aa, Camelus bactrianus
QVQLQESGGGSVQAGGSLKLSCVVS

SEQ ID NO: 40 - protein, 25 aa, Camelus bactrianus
QVQLQESGGGSVQAGGSLRLSCAAS

SEQ ID NO: 41 - protein, 25 aa, Camelus bactrianus
QVQLQESGGGSVQPGGSLRLSCVVS

SEQ ID NO: 42 - protein, 25 aa, Camelus bactrianus
QVQLQESGGGSVQPGGSLRLSCVAS

SEQ ID NO: 43 - protein, 14 aa, Camelus bactrianus
WFRQTPGKEREGVA

SEQ ID NO: 44 - protein, 14 aa, Camelus bactrianus
WFRQAPGKEREGVA

SEQ ID NO: 45 - protein, 14 aa, Camelus bactrianus
WFRQAPGMERELVA

SEQ ID NO: 46 - protein, 14 aa, Camelus bactrianus
WVRQAPGKGLEWVS

SEQ ID NO: 47 - protein, 14 aa, Camelus bactrianus
WFRQAPGKERELVA

SEQ ID NO: 48 - protein, 40 aa, Camelus bactrianus
KYAGSVKGRFTMSRDNAKNTLLLQMNSLKPEDTAIYYCAA

SEQ ID NO: 49 - protein, 40 aa, Camelus bactrianus
TYKPSVEGRFTISRDSAKRTLYLQMNSLKPEDTAMYYCAT

SEQ ID NO: 50 - protein, 40 aa, Camelus bactrianus
TAADSVKGRFTISRDNAKNTLSLQMTSLKPEDTAMYYCAA

SEQ ID NO: 51 - protein, 40 aa, Camelus bactrianus
YYGDSVKGRFTASQDNAKNTLYLQMNSLKPEDTATYYCAR

SEQ ID NO: 52 - protein, 40 aa, Camelus bactrianus
FYAESVKGRFTMSTDNAKNTVYLQMTSLKPEDTAVYYCSP

SEQ ID NO: 53 - protein, 40 aa, Camelus bactrianus
YYAGSVKGRFTISQEHATNTLYLQMNSLKPEDTAMYYCAA

SEQ ID NO: 54 - protein, 11 aa, Camelus bactrianus
WGQGTQVTVSS

SEQ ID NO: 55 - protein, 11 aa, Camelus bactrianus
RGQGTQVTVSS